European Patent Application EP 4 400 113 A1, published July 17, 2024. Title: A Hypoxia-triggered Artificial Transcription Factor, a Hypoxia-triggered Transcription Control System and Use Thereof. Applicant: SHANGHAI SINOBAY BIOTECHNOLOGY CO., LTD. Application EP21953423.7. The sequence listing filed with the application follows.

SEQUENCE LISTING (9 sequences)

SEQ ID NO: 1 - protein, 661 aa, Artificial Sequence
  Hypoxia-triggered Artificial Transcription Factor (HATF)
MHHHHHHPKKKRKVSNLLTVHQNLPALPVDATSDEVRKNLMDMFRDRQAFSEHTWKMLLSVCRSWAAWCKLNNRKWFPAEPEDVRDYLLYLQARGLAVKTIQQHLGQLNMLHRRSGLPRPSDSNAVSLVMRRIRKENVDAGERAKQALAFERTDFDQVRSLMENSDRCQDIRNLAFLGIAYNTLLRIAEIARIRVKDISRTDGGRMLIHIGRTKTLVSTAGVEKALSLGVTKLVERWISVSGVADDPNNYLFCRVRKNGVAAPSATSQLSTRALEGIFEATHRLIYGAKDDSGQRYLAWSGHSARVGAARDMARAGVSIPEIMQAGGWTNVNIVMNFIRNLDSETGAMVRLLEDGDSRAAAGGSGGSGGSDALDDFDLDMLGSDALDDFDLDMLGSDALDDFDLDMLGSDALDDFDLDMLGSGGGGSGGGGSGGGGSSEDTSSLFDKLKKEPDALTLLAPAAGDTIISLDFGSNDTETDDQQLEEVPLYNDVMLPSPNEKLQNINLAMSPLPTAETPKPLRSSADPALNQEVALKLEPNPESLELSFTMPQIQDQTPSPSDGSTRQSSPEPNSPSEYCFYVDSDMVNEFKLELVEKLFAEDTEAKNPFSTQDTDLDLEMLAPYIPMDDDFQLRSFDQLSPLESSSASPESASPQSTVTVFQ

SEQ ID NO: 2 - DNA, 34 bp, Artificial Sequence
  Recognition element (RE)
ataacttcgtataatgtatgctatacgaagttat

SEQ ID NO: 3 - DNA, 269 bp, Artificial Sequence
  Recognition element (RE)
taacttcgtataatgtatgctatacgaagttatataacttcgtataatgtatgctatacgaagttatataacttcgtataatgtatgctatacgaagttataaagtgaaagtcgagctcggtacccgggtcgactgcatataagcagctgctctgcatataagcagctgctttttgcctgtactgggtctctctggttagaccagatctgagcctgggagctctctggctaactagggaacccactgcttaagcctcaataaagcttgc

SEQ ID NO: 4 - DNA, 35 bp, Artificial Sequence
  Hypoxia-triggered Transcription Reaction Element (HRTE)
ccacagtgcatacgtgggctccaacaggtcctctt

SEQ ID NO: 5 - DNA, 175 bp, Artificial Sequence
  Hypoxia-triggered Transcription Reaction Element (HRTE)
ccacagtgcatacgtgggctccaacaggtcctcttccacagtgcatacgtgggctccaacaggtcctcttccacagtgcatacgtgggctccaacaggtcctcttccacagtgcatacgtgggctccaacaggtcctcttccacagtgcatacgtgggctccaacaggtcctctt

SEQ ID NO: 6 - protein, 236 aa, Artificial Sequence
  Red Fluorescent Protein mCherry
MVSKGEEDNMAIIKEFMRFKVHMEGSVNGHEFEIEGEGEGRPYEGTQTTKLKVTKGGPLPFAWDILSPQFMYGSKAYVKHPADIPDYLKLSFPEGFKWERVMNFEDGGVVTVTQDSSLQDGEFIYKVKLRGTNFPSDGPVMQKKTMGWEASSERMYPEDGALKGEIKQRLKLKDGGHYDAEVKTTYKAKKPVQLPGAYNVNIKLDITSHNEDYTIVEQYERAEGRHSTGGMDELYK

SEQ ID NO: 7 - protein, 498 aa, Artificial Sequence
  Chimeric Antigen Receptor (CAR) Binding to Tumor Antigen HER2
MALPVTALLLPLALLLHAARPDYKDDDDKDIQMTQSPSSLSASVGDRVTITCRASQDVNTAVAWYQQKPGKAPKLLIYSASFLYSGVPSRFSGSRSGTDFTLTISSLQPEDFATYYCQQHYTTPPTFGQGTKVEIKRTGSTSGSGKPGSGEGSEVQLVESGGGLVQPGGSLRLSCAASGFNIKDTYIHWVRQAPGKGLEWVARIYPTNGYTRYADSVKGRFTISADTSKNTAYLQMNSLRAEDTAVYYCSRWGGDGFYAMDVWGQGTLVTVSSTRTTTPAPRPPTPAPTIASQPLSLRPEACRPAAGGAVHTRGLDFACDIYIWAPLAGTCGVLLLSLVITLYCKRGRKKLLYIFKQPFMRPVQTTQEEDGCSCRFPEEEEGGCELRVKFSRSADAPAYKQGQNQLYNELNLGRREEYDVLDKRRGRDPEMGGKPRRKNPQEGLYNELQKDKMAEAYSEIGMKGERRRGKGHDGLYQGLSTATKDTYDALHMQALPPR

SEQ ID NO: 8 - protein, 520 aa, Artificial Sequence
  Bispecific T-cell Engager (BiTE) of CD47/CD3
MGWSCIILFLVATATGEIVLTQSPATLSLSPGERATLSCRASQTISDYLHWYQQKPGQAPRLLIKFASQSISGIPARFSGSGSGTDFTLTISSLEPEDFAVYYCQNGHGFPRTFGQGTKVEIKGGGGSGGGGSGGGGSQVQLVQSGAEVKKPGASVKVSCKASGYTFTRYTMHWVRQAPGQGLEWMGYINPSRGYTNYNQKFKDRVTITADKSTSTAYMELSSLRSEDTAVYYCARYYDDHYCLDYWGQGTTVTVSSGGGGSGGGGSGGGGSGSEIVLTQSPATLSLSPGERATLSCSASSSVSYMNWYQQKPGKAPKRLIYDTSKLASGVPSRFSGSGSGTDFTLTINSLEAEDAATYYCQQWSSNPFTFGQGTKVEIKRGGGGSGGGGSGGGGSEVQLVESGGGLVQPGGSLRLSCAASGFTFSGYGMSWVRQAPGKGLEWVATITSGGTYTYYPDSVKGRFTISRDNAKNSLYLQMNSLRAEDTAVYYCARSLAGNAMDYWGQGTLVTVSSHHHHHH

SEQ ID NO: 9 - DNA, 2539 bp, Artificial Sequence
  Hypoxia-Triggered Transcription Control System
tcactggaacacggtcacggttgactgtggtgaagcgctctcaggacttgcgctagaagattcgagaggggacagctgatcaaatgaccgcagctgaaagtcatcgtccataggaatgtaaggtgcgagcatttctaagtccaggtcggtgtcctgtgttgaaaatgggttctttgcctcagtatcctctgcgaacagcttctcgactaactccagcttaaactcattcaccatgtcgctatcgacgtagaagcagtactcggatggggaattgggctcaggggaagactgcctagttgatccgtcggatggagatggagtctgatcctgaatctgtggcatagtaaatgaaagctccagagactctgggtttggctctagcttcagggccacctcctggttcagagcgggatcggcgctagacctgagtggcttaggtgtctcggcggtaggcagtggtgacatagccagattaatattttgcagcttctcattaggagaaggcagcatgacatcattgtacagaggcacctcctccagctgctggtcgtcggtctctgtatcgttagacccaaagtccaggctaataattgtatcgccggcggcgggtgcgaggagtgtgagtgcgtcgggctccttcttgagcttgtcaaacagtgatgaggtatcctcgctggaccctccgccgccggagcccccgcccccggacccgcctccgcctgatccgagcatgtccaggtcaaagtcatccagtgcatctgatcccaacatgtcgagatcgaaatcgtccagagcgtcagatcccagcatgtccagatcaaaatcatccagggcgtcgctgcccagcatatccaggtcgaagtcgtccagggcatcagatccgccagagcctccgcttccgcctgcggcagctctagaatcgccgtcctcgagcaggcgcaccatagccccggtctcagaatcgaggtttctgatgaagttcatcacaatattcacattggtccatccccctgcctgcataatctctgggatagagaccccggctctagccatatcgcgggcggctcccactctagctgagtggccggaccaagccaggtaccgctgcccgctatcgtccttggccccgtaaatgagtctgtgggttgcctcgaaaattccctccagtgccctagtagacagctgtgaagttgcagaaggggcagcgacgccgttcttccgcactctacaaaacaggtaattattagggtcgtcggcgacgccggacacgctaatccaccgctcgaccagctttgtcactcccagtgacagagccttctcgacgccagcagtagacacgagtgtctttgtgcgtccgatgtggatgagcatgcgccctccgtcagtgcgtgaaatatccttgactctgatcctagcgatctctgcaatgcgcaggagggtgttgtatgcaattcccagaaaggcgagattccgaatgtcctggcaccgatcagagttctccatgagggatctcacctgatcaaagtcggtccgctcaaaggcgagggcctgcttagcgcgctcgccagcgtcgacgttctcctttctaatgcgtctcatgacgagtgacacggcattggaatcagatggtctagggaggccggaccggcggtggagcatgttcagctggccgaggtgctgctgaatagtcttgactgccagtcccctagcctggaggtacagcaggtagtcgcgcacatcctcgggctcggctgggaaccacttgcggttattgagcttacaccaagcggcccaagacctacacacggacaggagcatcttccaagtgtgctcgctaaaagcctgtctatcgcgaaacatatccatgagattcttccgcacctcatcggaagttgcatccacggggagagcgggcagattctggtggactgtcaggagattagagaccttgcgcttcttcttagggtggtggtggtggtggtgcatctgcagaccggtggatcccagcacagtctccaggcgatctgacggttcactaaacgagctctgcttatataggcctcccaccgtacacgccacctcgacataccacagtgcatacgtgggctccaacaggtcctcttccacagtgcatacgtgggctccaacaggtcctcttccacagtgcatacgtgggctccaacaggtcctcttccacagtgcatacgtgggctccaacaggtcctcttccacagtgcatacgtgggctccaacaggtcctcttatgcatataacttcgtataatgtatgctatacgaagttatataacttcgtataatgtatgctatacgaagttatataacttcgtataatgtatgctatacgaagttataaagtgaaagtcgagctcggtacccgggtcgactgcatataagcagctgctctgcatataagcagctgctttttgcctgtactgggtctctctggttagaccagatctgagcctgggagctctctggctaactagggaacccactgcttaagcctcaataaagcttgc